European Patent Specification EP 3 957 318 B1, published August 21, 2024. Title: Medical Composition. Applicant: Hirata Corporation. The sequence listing filed with the application follows.

SEQUENCE LISTING (2 sequences)

SEQ ID NO: 1 - protein, 70 aa, Human
ASLAADTPTACCFSYTSRQIPQNFIADYFETSSQCSKPGVIFLTKRSRQVCADPSEEWVQKYVSDLELSA

SEQ ID NO: 2 - protein, 69 aa, Artificial Sequence
  Variant of CCL3
SLAADTPTACCFSYTSRQIPQNFIAAYFETSSQCSKPGVIFLTKRSRQVCADPSEEWVQKYVSDLELSA